European Patent Application EP 4 566 596 A1, published June 11, 2025. Title: Anti HBV agent. Applicant: Riken. Application JP. The sequence listing filed with the application follows.

SEQUENCE LISTING (11 sequences)

SEQ ID NO: 1 - DNA, 20 bp, HBV
  source 1..20: mol_type = other DNA
actcaccaacctcctgtcct

SEQ ID NO: 2 - DNA, 20 bp, HBV
  source 1..20: mol_type = other DNA
gacaaacgggcaacatacct

SEQ ID NO: 3 - DNA, 24 bp, HBV
  source 1..24: mol_type = other DNA
tatcgctggatgtgtctgcggcgt

SEQ ID NO: 4 - RNA, 23 nt, HBV
  source 1..23: mol_type = other RNA
ctcaatctcgggaatctcaatgt

SEQ ID NO: 5 - RNA, 23 nt, HBV
  source 1..23: mol_type = other RNA
ggatagaacctagcaggcataat

SEQ ID NO: 6 - RNA, 21 nt, HBV
  source 1..21: mol_type = other RNA
cacatcaggattcctaggacc

SEQ ID NO: 7 - RNA, 20 nt, HBV
  source 1..20: mol_type = other RNA
aggttggtgagtgattggag

SEQ ID NO: 8 - RNA, 26 nt, HBV
  source 1..26: mol_type = other RNA
cagagtctagactcgtggtggacttc

SEQ ID NO: 9 - DNA, 19 bp, HBV
  source 1..19: mol_type = other DNA
gtggctatcctgccttaat

SEQ ID NO: 10 - DNA, 18 bp, HBV
  source 1..18: mol_type = other DNA
cagagctgaggcggtgtc

SEQ ID NO: 11 - DNA, 25 bp, synthetic construct
  source 1..25: mol_type = other DNA
agttggcgagaaagtgaaagcctgc